European Patent Specification EP 3 322 729 B1, published September 9, 2026. Title: ANTIBODY MOLECULES WHICH BIND CD45. Applicant: UCB BIOPHARMA SPRL. The sequence listing filed with the application follows.

SEQUENCE LISTING (215 sequences)

SEQ ID NO: 1 - protein, 11 aa, Artificial Sequence
  CDRH1 formula
  misc_feature (2)..(2): Xaa is F or V
  misc_feature (6)..(6): Xaa is S, G or A
  misc_feature (7)..(7): Xaa is G, S or N
  misc_feature (9)..(9): Xaa is W or Y
  misc_feature (10)..(10): Xaa is I or M
  misc_feature (11)..(11): Xaa is C, S or Y
GXSFSXXYXXX

SEQ ID NO: 2 - protein, 18 aa, Artificial Sequence
  CDRH2 formula
  misc_feature (1)..(1): Xaa can be amino acid C or S
  misc_feature (2)..(2): Xaa can be amino acid T, I or L
  misc_feature (4)..(4): Xaa can be amino acid A or T
  misc_feature (6)..(6): Xaa can be amino acid R or S
  misc_feature (14)..(14): Xaa can be amino acid N or S
  misc_feature (16)..(16): Xaa can be amino acid V or A
  misc_feature (17)..(17): Xaa can be amino acid N or K
  misc_feature (18)..(18): Xaa can be amino acid G, A, S or T
XXYXGXSGSTYYAXWXXX

SEQ ID NO: 3 - protein, 12 aa, Artificial Sequence
  CDRH3 formula
  misc_feature (1)..(1): Xaa can be amino acid G, A or D
  misc_feature (2)..(2): Xaa can be amino acid N, S or L
  misc_feature (3)..(3): Xaa can be amino acid A or G
  misc_feature (4)..(4): Xaa can be amino acid G, W or Y
  misc_feature (5)..(5): Xaa can be amino acid V, T or E
  misc_feature (6)..(6): Xaa can be amino acid I or absent
  misc_feature (7)..(7): Xaa can be amino acid D or absent
  misc_feature (8)..(8): Xaa can be amino acid G, S, A, T or Y
  misc_feature (9)..(9): Xaa can be amino acid Y, V or G
  misc_feature (10)..(10): Xaa can be amino acid G or M
  misc_feature (11)..(11): Xaa can be amino acid G, A or D
XXXXXXXXXXXL

SEQ ID NO: 4 - protein, 13 aa, Artificial Sequence
  CDRL1 formula
  misc_feature (6)..(6): Xaa can be amino acid I, F or V
  misc_feature (7)..(7): Xaa can be amino acid S or Y
  misc_feature (8)..(8): Xaa can be amino acid N or S
  misc_feature (9)..(9): Xaa can be amino acid W, L or N
  misc_feature (10)..(10): Xaa can be amino acid N or absent
  misc_feature (11)..(11): Xaa can be amino acid N, S, Q or absent
  misc_feature (13)..(13): Xaa can be amino acid N  or A
QASQSXXXXXXLX

SEQ ID NO: 5 - protein, 7 aa, Artificial Sequence
  CDRL2 formula
  misc_feature (1)..(1): Xaa can be amino acid Q, G or D
  misc_feature (4)..(4): Xaa can be amino acid K, N or D
XASXLAS

SEQ ID NO: 6 - protein, 13 aa, Artificial Sequence
  CDRL3 formula VI
  misc_feature (1)..(1): Xaa can be amino acid Q or  absent
  misc_feature (2)..(2): Xaa can be amino acid S or L
  misc_feature (3)..(3): Xaa can be amino acid S or L
  misc_feature (4)..(4): Xaa can be amino acid Y, G or absent
  misc_feature (5)..(5): Xaa can be amino acid D or Y
  misc_feature (6)..(6): Xaa can be amino acid G, A, T, S or Y
  misc_feature (7)..(7): Xaa can be amino acid G or S
  misc_feature (9)..(9): Xaa can be amino acid N, S, Y or G
  misc_feature (10)..(10): Xaa can be amino acid V, A or W
  misc_feature (11)..(11): Xaa can be amino acid F or Y or absent
  misc_feature (12)..(12): Xaa can be amino acid F or absent
  misc_feature (13)..(13): Xaa can be amino acid N, A or absent
XXXXXXXSXXXXX

SEQ ID NO: 7 - protein, 11 aa, Artificial Sequence
  CDRH1 formula Ia
  misc_feature (6)..(6): Xaa can be amino acid S, G or A
  misc_feature (7)..(7): Xaa can be amino acid G, S or N
  misc_feature (9)..(9): Xaa can be amino acid W or Y
  misc_feature (10)..(10): Xaa can be amino acid I or M
  misc_feature (11)..(11): Xaa can be amino acid C, S or Y
GFSFSXXYXXX

SEQ ID NO: 8 - protein, 11 aa, Artificial Sequence
  CDRH1 formula Ib
  misc_feature (6)..(6): Xaa can be amino acid S, G or A
  misc_feature (7)..(7): Xaa can be amino acid G, S or N
  misc_feature (11)..(11): Xaa can be amino acid C, S or Y
GFSFSXXYWIX

SEQ ID NO: 9 - protein, 13 aa, Artificial Sequence
  CDRL1 formula VIa
  misc_feature (3)..(3): Xaa can be amino acid Y, A or G
  misc_feature (6)..(6): Xaa can be amino acid G, A, T, S or Y
  misc_feature (7)..(7): Xaa can be amino acid G or S
  misc_feature (9)..(9): Xaa can be amino acid N, S, Y or G
  misc_feature (10)..(10): Xaa can be amino acid V, A or W
  misc_feature (11)..(11): Xaa can be amino acid F or Y or absent
  misc_feature (12)..(12): Xaa can be amino acid F or absent
  misc_feature (13)..(13): Xaa can be amino acid N, A or absent
QSXYDXXSXXXXX

SEQ ID NO: 10 - protein, 11 aa, Artificial Sequence
  CDRH1
GFSFSAGYWIC

SEQ ID NO: 11 - protein, 11 aa, Artificial Sequence
  CDRH1
GFSFSAGYWIS

SEQ ID NO: 12 - protein, 11 aa, Artificial Sequence
  CDRH1
GFSFSAGYWIC

SEQ ID NO: 13 - protein, 11 aa, Artificial Sequence
  CDRH1
GFSFSAGYWIS

SEQ ID NO: 14 - protein, 11 aa, Artificial Sequence
  CDRH1
GVSFSSSYWIY

SEQ ID NO: 15 - protein, 11 aa, Artificial Sequence
  CDRH1
GFSFSGNYYMC

SEQ ID NO: 16 - protein, 11 aa, Artificial Sequence
  CDRH1
GFSFSGNYYMS

SEQ ID NO: 17 - protein, 18 aa, Artificial Sequence
  CDRH2
CTYAGRSGSTYYANWVNG

SEQ ID NO: 18 - protein, 18 aa, Artificial Sequence
  CDRH2
CTYAGRSGSTYYANWVNA

SEQ ID NO: 19 - protein, 18 aa, Artificial Sequence
  CDRH2
CTYAGRSGSTYYANWVNS

SEQ ID NO: 20 - protein, 18 aa, Artificial Sequence
  CDRH2
CTYAGRSGSTYYANWVNT

SEQ ID NO: 21 - protein, 18 aa, Artificial Sequence
  CDRH2
STYAGRSGSTYYANWVNG

SEQ ID NO: 22 - protein, 18 aa, Artificial Sequence
  CDRH2
STYAGRSGSTYYANWVNA

SEQ ID NO: 23 - protein, 18 aa, Artificial Sequence
  CDRH2
STYAGRSGSTYYANWVNS

SEQ ID NO: 24 - protein, 18 aa, Artificial Sequence
  CDRH2
STYAGRSGSTYYANWVNT

SEQ ID NO: 25 - protein, 18 aa, Artificial Sequence
  CDRH2
CIYAGSSGSTYYASWAKG

SEQ ID NO: 26 - protein, 18 aa, Artificial Sequence
  CDRH2
SIYAGSSGSTYYASWAKG

SEQ ID NO: 27 - protein, 18 aa, Artificial Sequence
  CDRH2
CIYTGSSGSTYYASWAKG

SEQ ID NO: 28 - protein, 18 aa, Artificial Sequence
  CDRH2
SIYTGSSGSTYYASWAKG

SEQ ID NO: 29 - protein, 18 aa, Artificial Sequence
  CDRH2
CLYTGSSGSTYYASWAKG

SEQ ID NO: 30 - protein, 18 aa, Artificial Sequence
  CDRH2
SLYTGSSGSTYYASWAKG

SEQ ID NO: 31 - protein, 10 aa, Artificial Sequence
  CDRH3
GNAGVAVGAL

SEQ ID NO: 32 - protein, 10 aa, Artificial Sequence
  CDRH3
GNAGVAVGAL

SEQ ID NO: 33 - protein, 10 aa, Artificial Sequence
  CDRH3
ASAWTYGMDL

SEQ ID NO: 34 - protein, 12 aa, Artificial Sequence
  CDRH3
DLGYEIDGYGGL

SEQ ID NO: 35 - protein, 12 aa, Artificial Sequence
  CDRH3
DLGYEIDSYGGL

SEQ ID NO: 36 - protein, 12 aa, Artificial Sequence
  CDRH3
DLGYEIDAYGGL

SEQ ID NO: 37 - protein, 12 aa, Artificial Sequence
  CDRH3
DLGYEIDTYGGL

SEQ ID NO: 38 - protein, 11 aa, Artificial Sequence
  CDRL1
QASQSISNWLA

SEQ ID NO: 39 - protein, 11 aa, Artificial Sequence
  CDRL1
QASQSISSWLS

SEQ ID NO: 40 - protein, 11 aa, Artificial Sequence
  CDRL1
QASQSFYNLLA

SEQ ID NO: 41 - protein, 13 aa, Artificial Sequence
  CDRL1
QASQSVYNNNNLS

SEQ ID NO: 42 - protein, 13 aa, Artificial Sequence
  CDRL1
QASQSVYNNNSLS

SEQ ID NO: 43 - protein, 13 aa, Artificial Sequence
  CDRL1
QASQSVYNNNQLS

SEQ ID NO: 44 - protein, 13 aa, Artificial Sequence
  CDRL1
QASQSVYNNNNLA

SEQ ID NO: 45 - protein, 7 aa, Artificial Sequence
  CDRL2
QASKLAS

SEQ ID NO: 46 - protein, 7 aa, Artificial Sequence
  CDRL2
GASNLAS

SEQ ID NO: 47 - protein, 7 aa, Artificial Sequence
  CDRL2
DASDLAS

SEQ ID NO: 48 - protein, 7 aa, Artificial Sequence
  CDRL2
DASKLAS

SEQ ID NO: 49 - protein, 13 aa, Artificial Sequence
  CDRL3
QSYYDSGSNVFFA

SEQ ID NO: 50 - protein, 13 aa, Artificial Sequence
  CDRL3
QSYYDAGSNVFFA

SEQ ID NO: 51 - protein, 13 aa, Artificial Sequence
  CDRL3
QSYYDTGSNVFFA

SEQ ID NO: 52 - protein, 13 aa, Artificial Sequence
  CDRL3
QSYYDSGSSVFFN

SEQ ID NO: 53 - protein, 13 aa, Artificial Sequence
  CDRL3
QSYYDAGSSVFFN

SEQ ID NO: 54 - protein, 13 aa, Artificial Sequence
  CDRL3
QSYYDTGSSVFFN

SEQ ID NO: 55 - protein, 9 aa, Artificial Sequence
  CDRL3
QSADGSSYA

SEQ ID NO: 56 - protein, 9 aa, Artificial Sequence
  CDRL3
QSADSSSYA

SEQ ID NO: 57 - protein, 9 aa, Artificial Sequence
  CDRL3
QSADASSYA

SEQ ID NO: 58 - protein, 9 aa, Artificial Sequence
  CDRL3
QSADTSSYA

SEQ ID NO: 59 - protein, 12 aa, Artificial Sequence
  CDRL3
LGGYYSSGWYFA

SEQ ID NO: 60 - protein, 111 aa, Artificial Sequence
  Rabbit Ab 4122 VL region
DIVMTQTPASVSEPVGGTVTIMCQASQSISNWLAWYQQKPGQPPKLLIYQASKLASGVPSRFKGSGSGTEYTLTISDLECADAATYYCQSYYDSGSNVFFAFGGGTKVVVE

SEQ ID NO: 61 - DNA, 333 bp, Artificial Sequence
  Rabbit Ab 4122 VL region
gacattgtgatgacccagactccagcctccgtgtctgaacctgtgggaggcacagtcaccatcatgtgccaggccagtcagagcattagcaattggttagcctggtatcaacagaaaccagggcagcctcccaagctcctgatctaccaggcatccaaactggcatctggggtcccatcgcggttcaaaggcagtggatctgggacagagtacactctcaccatcagcgacctggagtgtgccgatgctgccacttactactgtcaaagctattatgatagtggtagtaatgttttttttgctttcggcggagggaccaaggtggtggtcgaa

SEQ ID NO: 62 - protein, 119 aa, Artificial Sequence
  Rabbit Ab 4122 VH region
LSLEESGGDLVKPGASLTLTCTASGFSFSAGYWICWVRQAPGKGLEWIACTYAGRSGSTYYANWVNGRFTIPKTSSTTVTLQMTSLSGADTASYFCARGNAGVAVGALWGPGTLVTVSS

SEQ ID NO: 63 - DNA, 357 bp, Artificial Sequence
  Rabbit Ab 4122 VH region
ctgtcgttggaggagtccgggggagacctggtcaagcctggggcatccctgacactcacctgcacagcctctggattctccttcagtgccggctattggatatgttgggtccgccaggctccagggaaggggctggagtggatcgcatgcacttatgctggtcgtagtggtagcacttactacgcgaactgggtgaatggccgattcaccatccccaaaacctcgtcgaccacggtgactctgcaaatgaccagtctgtcaggcgcggacacggccagctatttctgtgcgagaggtaatgctggtgttgctgttggtgccttgtggggcccaggcaccctggtcaccgtctcgagt

SEQ ID NO: 64 - protein, 111 aa, Artificial Sequence
  4122 gL1 V-region - IGKV1-5 framework
DIQMTQSPSTLSASVGDRVTITCQASQSISNWLAWYQQKPGKAPKLLIYQASKLASGVPSRFSGSGSGTEYTLTISSLQPDDFATYYCQSYYDSGSNVFFAFGGGTKVEIK

SEQ ID NO: 65 - protein, 121 aa, Artificial Sequence
  4122 gH6 V-region - IGHV3-7 framework
EVQLVESGGGLVQPGGSLRLSCAASGFSFSAGYWICWVRQAPGKGLEWIACTYAGRSGSTYYANWVNGRFTISKDSAKTSVYLQMNSLRAEDTAVYYCARGNAGVAVGALWGRGTLVTVSS

SEQ ID NO: 66 - protein, 121 aa, Artificial Sequence
  4122 gH4 V-region - IGHV3-7 framework
EVQLVESGGGLVQPGGSLRLSCAASGFSFSAGYWISWVRQAPGKGLEWIASTYAGRSGSTYYANWVNGRFTISKDSAKTSVYLQMNSLRAEDTAVYYCARGNAGVAVGALWGRGTLVTVSS

SEQ ID NO: 67 - protein, 121 aa, Artificial Sequence
  4122 gH3 V-region - IGHV2-70 framework
EVTLKESGPALVKPTQTLTLTCTASGFSFSAGYWICWVRQPPGKGLEWIACTYAGRSGSTYYANWVNGRFTISKDSSKTQVVLTMTNMDPVDTATYYCARGNAGVAVGALWGRGTLVTVSS

SEQ ID NO: 68 - protein, 121 aa, Artificial Sequence
  4122 gH5 V-region - IGHV2-70 framework
EVTLKESGPALVKPTQTLTLTCTASGFSFSAGYWISWVRQPPGKGLEWIASTYAGRSGSTYYANWVNGRFTISKDSSKTQVVLTMTNMDPVDTATYYCARGNAGVAVGALWGRGTLVTVSS

SEQ ID NO: 69 - protein, 111 aa, Artificial Sequence
  Rabbit Ab 4129 VL region
DIVMTQTPASVEAAVGGTVTINCQASQSISSWLSWYQQKPGQPPKLLIYGASNLASGVPSRFSGSGSGTQFSLTISDLECADAATYYCQSYYDSGSSVFFNFGGGTKVVVK

SEQ ID NO: 70 - DNA, 333 bp, Artificial Sequence
  Rabbit Ab 4129 VL region
gacattgtgatgacccagactccagcctccgtggaggcagctgtgggaggcacagtcaccatcaattgccaagccagtcagagcattagcagttggttatcctggtatcagcagaaaccagggcagcctcccaagctcctgatctatggtgcatccaatctggcatctggggtcccatcacggttcagcggcagtggatctgggacacagttcagtctcaccatcagcgacctggagtgtgccgatgctgccacttactactgtcaaagctattatgatagtggtagtagtgttttttttaatttcggcggagggaccaaggtggtcgtcaaa

SEQ ID NO: 71 - protein, 119 aa, Artificial Sequence
  Rabbit Ab 4129 VH region
QSLEESGGDLVKPGASLTLTCTASGFSFSAGYWICWVRQAPGKGLEWIACIYAGSSGSTYYASWAKGRFTIPKTSSTTVTLQMTSLTGADTATYFCARGNAGVAVGALWGPGTLVTVSS

SEQ ID NO: 72 - DNA, 357 bp, Artificial Sequence
  Rabbit Ab 4129 VH region
cagtcgttggaggagtccgggggagacctggttaagcctggggcatccctgacactcacctgcacagcctctggattctccttcagtgccggctattggatatgttgggtccgccaggctccagggaaggggctggagtggatcgcatgcatttatgctggtagtagtggtagcacttactacgcgagctgggcgaaaggccgattcaccatccccaaaacctcgtcgaccacggtgactctgcaaatgaccagtctgacaggcgcggacacggccacctatttctgtgcgagaggtaatgctggtgttgctgttggtgccttgtggggcccaggcaccctcgtcaccgtctcgagt

SEQ ID NO: 73 - protein, 111 aa, Artificial Sequence
  4129 gL3 V-region - IGKV1-5 framework
DIQMTQSPSTLSASVGDRVTITCQASQSISSWLSWYQQKPGKAPKLLIYGASNLASGVPSRFSGSGSGTQFTLTISSLQPDDFATYYCQSYYDSGSSVFFNFGGGTKVEIK

SEQ ID NO: 74 - protein, 121 aa, Artificial Sequence
  4129 gH1 V-region - IGHV3-7 framework
EVQLVESGGGLVQPGGSLRLSCAASGFSFSAGYWICWVRQAPGKGLEWIACIYAGSSGSTYYASWAKGRFTISKDSAKTSVYLQMNSLRAEDTAVYYCARGNAGVAVGALWGRGTLVTVSS

SEQ ID NO: 75 - protein, 121 aa, Artificial Sequence
  4129 gH4 V-region - IGHV3-7 framework
EVQLVESGGGLVQPGGSLRLSCAASGFSFSAGYWISWVRQAPGKGLEWIASIYAGSSGSTYYASWAKGRFTISKDSAKTSVYLQMNSLRAEDTAVYYCARGNAGVAVGALWGRGTLVTVSS

SEQ ID NO: 76 - protein, 121 aa, Artificial Sequence
  4129 gH3 V-region - IGHV2-70 framework
EVTLKESGPALVKPTQTLTLTCTASGFSFSAGYWICWVRQPPGKGLEWIACIYAGSSGSTYYASWAKGRFTISKDSSKTQVVLTMTNMDPVDTATYYCARGNAGVAVGALWGRGTLVTVSS

SEQ ID NO: 77 - protein, 121 aa, Artificial Sequence
  4129 gH5 V-region - IGHV2-70 framework
EVTLKESGPALVKPTQTLTLTCTASGFSFSAGYWISWVRQPPGKGLEWIASIYAGSSGSTYYASWAKGRFTISKDSSKTQVVLTMTNMDPVDTATYYCARGNAGVAVGALWGRGTLVTVSS

SEQ ID NO: 78 - protein, 107 aa, Artificial Sequence
  Rabbit Ab 4131 VL region
DIVMTQTPASVSEPVGGSVTIKCQASQSFYNLLAWYQQKPGQPPKLLIYDASDLASGVPSRFKGSGSGTDFTLTISDLECADAAAYYCQSADGSSYAFGGGTEVVVK

SEQ ID NO: 79 - DNA, 321 bp, Artificial Sequence
  Rabbit Ab 4131 VL region
gacattgtgatgacccagactccagcctccgtgtctgaacctgtgggaggctcagtcaccatcaagtgccaggccagtcagagcttttacaacctcttagcctggtatcagcagaaaccagggcagcctcccaaactcctgatctatgatgcatccgatctggcatctggggtcccatcgcggttcaaaggcagtggatctgggactgatttcactctcaccatcagcgacctggagtgtgccgatgctgccgcttactactgtcaaagtgctgatggtagtagttacgctttcggcggagggaccgaggtggtcgtcaaa

SEQ ID NO: 80 - protein, 120 aa, Artificial Sequence
  Rabbit Ab 4131 VH region
QEQLEESGGGLVKPEGSLTLTCTASGVSFSSSYWIYWVRQAPGKGLEWIACIYTGSSGSTYYASWAKGRFTVSETSSTTVTLQMTSLTAADTATYFCARASAWTYGMDLWGPGTLVTVSS

SEQ ID NO: 81 - DNA, 360 bp, Artificial Sequence
  Rabbit Ab 4131 VH region
caggagcaattggaggagtccgggggaggcctggtcaagcctgagggatccctgacactcacctgcacagcctctggagtctccttcagtagcagctattggatatactgggtccgccaggctccagggaaggggctggagtggatcgcatgcatttatactggtagtagtggtagcacttactacgcgagctgggcgaaaggccgattcaccgtctccgaaacctcgtcgaccacggtgactctgcaaatgaccagtctgacagccgcggacacggccacctatttctgtgcgagagcaagcgcttggacctacggcatggacctctggggcccgggcaccctcgtcaccgtctcgagt

SEQ ID NO: 82 - protein, 107 aa, Artificial Sequence
  4131 gL8 V-region - IGKV1-12 framework
DIVMTQSPSSVSASVGDRVTITCQASQSFYNLLAWYQQKPGKAPKLLIYDASDLASGVPSRFKGSGSGTDFTLTISSLQPEDFATYYCQSADGSSYAFGGGTKVEIK

SEQ ID NO: 83 - protein, 107 aa, Artificial Sequence
  4131 gL3 V-region - IGKV1-12 framework
DIQMTQSPSSVSASVGDRVTITCQASQSFYNLLAWYQQKPGKAPKLLIYDASDLASGVPSRFSGSGSGTDFTLTISSLQPEDFATYYCQSADGSSYAFGGGTKVEIK

SEQ ID NO: 84 - protein, 121 aa, Artificial Sequence
  4131 gH5 V-region - IGHV3-7 framework
EVQLVESGGGLVQPGGSLRLSCAASGVSFSSSYWIYWVRQAPGKGLEWIACIYTGSSGSTYYASWAKGRFTVSEDSAKTSVYLQMNSLRAEDTAVYYCARASAWTYGMDLWGRGTLVTVSS

SEQ ID NO: 85 - protein, 121 aa, Artificial Sequence
  4131 gH4 V-region - IGHV3-7 framework
EVQLVESGGGLVQPGGSLRLSCAASGVSFSSSYWIYWVRQAPGKGLEWIASIYTGSSGSTYYASWAKGRFTVSEDSAKTSVYLQMNSLRAEDTAVYYCARASAWTYGMDLWGRGTLVTVSS

SEQ ID NO: 86 - protein, 121 aa, Artificial Sequence
  4131 gH6 V-region - IGHV4-31 framework
EVQLQESGPGLVKPSQTLSLTCTASGVSFSSSYWIYWVRQHPGKGLEWIACIYTGSSGSTYYASWAKGRFTVSEDSSKTQVSLKLSSVTAADTAVYYCARASAWTYGMDLWGRGTLVTVSS

SEQ ID NO: 87 - protein, 121 aa, Artificial Sequence
  4131 gH3 V-region - IGHV4-31 framework
EVQLQESGPGLVKPSQTLSLTCTASGVSFSSSYWIYWVRQHPGKGLEWIASIYTGSSGSTYYASWAKGRFTVSEDSSKTQVSLKLSSVTAADTAVYYCARASAWTYGMDLWGRGTLVTVSS

SEQ ID NO: 88 - protein, 112 aa, Artificial Sequence
  Rabbit Ab 4133 VL region
AQVLTQTPSPVSAVVGGTVSISCQASQSVYNNNNLSWYQQKPGQPPKLLIYDASKLASGVPSRFKGSGSGTQFTLTISGVQCDDAATYYCLGGYYSSGWYFAFGGGTKVVVK

SEQ ID NO: 89 - DNA, 336 bp, Artificial Sequence
  Rabbit Ab 4133 VL region
gcgcaagtgctgacccagactccatctcccgtgtctgcagttgtgggaggcacagtcagcatcagttgccaggccagtcagagtgtttataataacaacaacttatcctggtatcagcagaaaccagggcagcctcccaagctcttgatctacgatgcatccaaattggcatctggggtcccatcccggttcaaaggcagtggatctgggacacagttcactctcaccatcagcggcgtgcagtgtgacgatgctgccacttactactgtctaggcggttattatagtagtggttggtattttgctttcggcggagggaccaaggtggtggtcaaa

SEQ ID NO: 90 - protein, 122 aa, Artificial Sequence
  Rabbit Ab 4133 VH region
QEQLVESGGGLVQPEGSLTLTCTASGFSFSGNYYMCWVRQAPGKGLEWIGCLYTGSSGSTYYASWAKGRFTISKTSSTTVTLQMTSLTAADTATYFCARDLGYEIDGYGGLWGQGTLVTVSS

SEQ ID NO: 91 - DNA, 366 bp, Artificial Sequence
  Rabbit Ab 4133 VH region
caggagcagctggtggagtccgggggaggcctggtccagcctgagggatccctgacactaacctgcacagcttctggattctccttcagtggcaactactacatgtgctgggtccgccaggctccagggaaggggctggagtggatcggatgcctttatactggtagtagtggtagcacatattacgcgagctgggcgaaaggccgattcaccatctccaaaacctcgtcgaccacggtgactctgcaaatgaccagtctgacagccgcggacacggccacctatttctgtgcgagagatctaggttatgaaattgatggttatgggggcttgtggggccagggcaccctcgtcaccgtctcgagt

SEQ ID NO: 92 - protein, 112 aa, Artificial Sequence
  4133 gL7 V-region - IGKV1D-13 framework
AQVLTQSPSSLSASVGDRVTITCQASQSVYNNNNLSWYQQKPGKAPKLLIYDASKLASGVPSRFSGSGSGTQFTLTISSLQPEDFATYYCLGGYYSSGWYFAFGGGTKVEIK

SEQ ID NO: 93 - protein, 112 aa, Artificial Sequence
  4133 gL1 V-region - IGKV1D-13 framework
AQVLTQSPSSLSASVGDRVTITCQASQSVYNNNNLAWYQQKPGKAPKLLIYDASKLASGVPSRFSGSGSGTQFTLTISSLQPEDFATYYCLGGYYSSGWYFAFGGGTKVEIK

SEQ ID NO: 94 - protein, 123 aa, Artificial Sequence
  4133 gH1 V-region - IGHV3-21 framework
EVQLVESGGGLVKPGGSLRLSCAASGFSFSGNYYMCWVRQAPGKGLEWIGCLYTGSSGSTYYASWAKGRFTISKDSAKTSVYLQMNSLRAEDTAVYYCARDLGYEIDGYGGLWGQGTLVTVSS

SEQ ID NO: 95 - protein, 123 aa, Artificial Sequence
  4133 gH4 V-region - IGHV3-21 framework
EVQLVESGGGLVKPGGSLRLSCAASGFSFSGNYYMSWVRQAPGKGLEWIGSLYTGSSGSTYYASWAKGRFTISKDSAKTSVYLQMNSLRAEDTAVYYCARDLGYEIDGYGGLWGQGTLVTVSS

SEQ ID NO: 96 - protein, 123 aa, Artificial Sequence
  4133 gH3 V-region - IGHV4-4 framework
EVQLQESGPGLVKPSGTLSLTCAASGFSFSGNYYMCWVRQPPGKGLEWIGCLYTGSSGSTYYASWAKGRVTISKDSSKTQVSLKLSSVTAADTAVYYCARDLGYEIDGYGGLWGQGTLVTVSS

SEQ ID NO: 97 - protein, 123 aa, Artificial Sequence
  4133 gH3 V-region - IGHV4-4 framework
EVQLQESGPGLVKPSGTLSLTCAASGFSFSGNYYMSWVRQPPGKGLEWIGSLYTGSSGSTYYASWAKGRVTISKDSSKTQVSLKLSSVTAADTAVYYCARDLGYEIDGYGGLWGQGTLVTVSS

SEQ ID NO: 98 - protein, 10 aa, Artificial Sequence
  CDRH1 Ab 4447
GFSLSNYAVS

SEQ ID NO: 99 - protein, 17 aa, Artificial Sequence
  CDRH2 Ab 4447
IIYIETGTTWYANWAKG

SEQ ID NO: 100 - protein, 17 aa, Artificial Sequence
  CDRH3 Ab 4447
EPYEPYDDSNIYYGMDP

SEQ ID NO: 101 - protein, 13 aa, Artificial Sequence
  CDRL1  Ab4447
QASQSVVSGNYLA

SEQ ID NO: 102 - protein, 7 aa, Artificial Sequence
  CDRL2 Ab4447
SASTLAS

SEQ ID NO: 103 - protein, 13 aa, Artificial Sequence
  CDRL3 Ab4447
LGEFSCSSHDCNA

SEQ ID NO: 104 - protein, 13 aa, Artificial Sequence
  CDRL3 Ab4447 variant 1
LGEFSSSSHDSNA

SEQ ID NO: 105 - protein, 13 aa, Artificial Sequence
  CDRL3 Ab4447  variant 2
LGEFSCSSHDSNA

SEQ ID NO: 106 - protein, 13 aa, Artificial Sequence
  CDRL3 Ab4447 variant 3
LGEFSSSSHDCNA

SEQ ID NO: 107 - protein, 113 aa, Artificial Sequence
  Rabbit Ab 4447 VL region
AQVLTQTPSPVSAPVGGTVTINCQASQSVVSGNYLAWLQQKPGQPPKQLIHSASTLASGVSSRFSGSGSGTQFTLTISGVQCEDAATYYCLGEFSCSSHDCNAFGGGTEVVVK

SEQ ID NO: 108 - DNA, 339 bp, Artificial Sequence
  Rabbit Ab 4447 VL region
gcccaagtgctgacccagactccgtcccctgtgtctgcacctgtgggaggcacagtcaccatcaattgccaggccagtcagagtgttgttagtggcaattacctagcctggcttcagcagaaaccagggcagcctcccaagcaactgatccattctgcatccactctggcatctggggtctcatcgcggttcagcggcagtggatctgggacacaattcactctcaccatcagcggcgtgcagtgtgaagatgctgccacttactactgtctaggcgaatttagttgtagtagtcatgattgtaatgctttcggcggagggaccgaggtggtggtcaaa

SEQ ID NO: 109 - protein, 123 aa, Artificial Sequence
  Rabbit Ab 4447 VH region
QSLEESGGRLVTPGTPLTLTCTVSGFSLSNYAVSWVRQAPGEGLEWIGIIYIETGTTWYANWAKGRFTISKTSTTVDLTITSPSTEDTATYFCAREPYEPYDDSNIYYGMDPWGPGTLVTVSS

SEQ ID NO: 110 - DNA, 369 bp, Artificial Sequence
  Rabbit Ab 4447 VH region
cagtcgctggaggagtccgggggtcgcctggtcacgcctgggacacccctgacactcacctgcaccgtctctggattctccctcagtaactatgcagtaagctgggtccgccaggctccaggggagggactggaatggatcgggatcatttatattgaaactggtaccacatggtacgcgaactgggcgaaaggccgattcaccatctccaaaacctcgaccacggtggatctgacaatcaccagtccgtcaaccgaggacacggccacctatttctgtgccagagaaccttatgaaccttatgatgatagtaatatttactacggcatggacccctggggcccaggcaccctcgtcaccgtctcgagt

SEQ ID NO: 111 - protein, 113 aa, Artificial Sequence
  4447 gL1 V-region - IGKV1D-13 framework
AQVLTQSPSSLSASVGDRVTITCQASQSVVSGNYLAWLQQKPGKAPKQLIHSASTLASGVPSRFSGSGSGTQFTLTISSLQPEDFATYYCLGEFSCSSHDCNAFGGGTKVEIK

SEQ ID NO: 112 - protein, 113 aa, Artificial Sequence
  4447 gL2 V-region - IGKV1D-13 framework
AQVLTQSPSSLSASVGDRVTITCQASQSVVSGNYLAWLQQKPGKAPKQLIHSASTLASGVPSRFSGSGSGTQFTLTISSLQPEDFATYYCLGEFSSSSHDSNAFGGGTKVEIK

SEQ ID NO: 113 - protein, 126 aa, Artificial Sequence
  4447 gH1 V-region - IGHV3-48 framework
EVQLVESGGGLVQPGGSLRLSCAVSGFSLSNYAVSWVRQAPGKGLEWIGIIYIETGTTWYANWAKGRFTISKDSAKNSVYLQMNSLRDEDTAVYYCAREPYEPYDDSNIYYGMDPWGQGTLVTVSS

SEQ ID NO: 114 - protein, 126 aa, Artificial Sequence
  4447 gH3 V-region - IGHV4-59 framework
EVQLQESGPGLVKPSETLSLTCTVSGFSLSNYAVSWVRQPPGKGLEWIGIIYIETGTTWYANWAKGRFTISKDSSKNQVSLKLSSVTAADTAVYYCAREPYEPYDDSNIYYGMDPWGQGTLVTVSS

SEQ ID NO: 115 - protein, 10 aa, Artificial Sequence
  CDRH1 Ab 4450
GFSLNNYVMV

SEQ ID NO: 116 - protein, 16 aa, Artificial Sequence
  CDRH2 Ab 4450
IIYVSGNAYYASWAKG

SEQ ID NO: 117 - protein, 12 aa, Artificial Sequence
  CDRH3 Ab 4450
DAGHSDVDVLDI

SEQ ID NO: 118 - protein, 13 aa, Artificial Sequence
  CDRL1 Ab 4450
QSSQSIYNNNDLA

SEQ ID NO: 119 - protein, 7 aa, Artificial Sequence
  CDRL2 Ab 4450
EASKLAS

SEQ ID NO: 120 - protein, 11 aa, Artificial Sequence
  CDRL3 Ab 4450
QGGGSGGDGIA

SEQ ID NO: 121 - protein, 11 aa, Artificial Sequence
  Ab 4450 CDRL3 - variant 1
QGGGSGGEGIA

SEQ ID NO: 122 - protein, 11 aa, Artificial Sequence
  Ab 4450 CDRL3 - variant 2
QGGGSGGDAIA

SEQ ID NO: 123 - protein, 11 aa, Artificial Sequence
  Ab 4450 CDRL3 - variant 3
QGGGSGGDSIA

SEQ ID NO: 124 - protein, 111 aa, Artificial Sequence
  Rabbit Ab 4450 VL region
AIDMTQTPSPVSAAVGGTVTINCQSSQSIYNNNDLAWYQQKPGQPPKLLIYEASKLASGVPSRFKGSGSGTQFTLTISGVQCDDAATYYCQGGGSGGDGIAFGGGTKVVVE

SEQ ID NO: 125 - DNA, 333 bp, Artificial Sequence
  Rabbit Ab 4450 VL region
gccattgatatgacccagactccatcccccgtgtctgcagctgtgggaggcacagtcaccatcaattgccagtccagtcagagtatttataataataatgacttagcctggtatcagcagaaaccagggcagcctcccaagctcctgatctacgaagcatccaaactggcatctggggtcccatcgcggttcaaaggcagtggatctgggacacagttcactctcaccatcagtggcgtgcagtgtgatgatgctgccacttactactgtcagggcggtggtagtggtggtgatggcattgctttcggcggagggaccaaggtggtcgtcgaa

SEQ ID NO: 126 - protein, 117 aa, Artificial Sequence
  Rabbit Ab 4450 VH region
QSVEESGGRLVTPGAPLTLTCTVSGFSLNNYVMVWVRQAPGKGLEWIGIIYVSGNAYYASWAKGRFTISRTSTTVDLKVTSLTTEDTATYFCARDAGHSDVDVLDIWGPGTLVTVSS

SEQ ID NO: 127 - DNA, 351 bp, Artificial Sequence
  Rabbit Ab 4450 VH region
cagtcggtggaggagtccgggggtcgcctggtcacgcctggggcacccctgacactcacctgcacagtctctggattctccctcaataactatgtaatggtctgggtccgccaggctccagggaaggggctggaatggatcggaatcatttatgttagtggtaatgcatactacgcgagctgggcaaaaggccgattcaccatctccagaacctcgaccacggtggatctgaaagtgaccagtctgacaaccgaggacacggccacctatttctgtgccagagatgctggtcatagtgatgtcgatgttttggatatttggggcccgggcaccctcgtcaccgtctcgagt

SEQ ID NO: 128 - protein, 111 aa, Artificial Sequence
  4450 gL1 V-region - IGKV1-6 framework
AIDMTQSPSSLSASVGDRVTITCQSSQSIYNNNDLAWYQQKPGKAPKLLIYEASKLASGVPSRFSGSGSGTQFTLTISSLQPEDFATYYCQGGGSGGDGIAFGGGTKVEIK

SEQ ID NO: 129 - protein, 120 aa, Artificial Sequence
  4450 gH1 V-region - IGHV3-66 framework
EVQLVESGGGLVQPGGSLRLSCAVSGFSLNNYVMVWVRQAPGKGLEWIGIIYVSGNAYYASWAKGRFTISRDSSKNTVYLQMNSLRAEDTAVYYCARDAGHSDVDVLDIWGQGTLVTVSS

SEQ ID NO: 130 - protein, 120 aa, Artificial Sequence
  4450 gH3 V-region - IGHV4-59 framework
EVQLQESGPGLVKPSETLSLTCTVSGFSLNNYVMVWVRQPPGKGLEWIGIIYVSGNAYYASWAKGRFTISRDSSKNQVSLKLSSVTAADTAVYYCARDAGHSDVDVLDIWGQGTLVTVSS

SEQ ID NO: 131 - protein, 10 aa, Artificial Sequence
  CDRH1 dAbH1
GIDLSNYAIN

SEQ ID NO: 132 - protein, 16 aa, Artificial Sequence
  CDRH2 dAbH1
IIWASGTTFYATWAKG

SEQ ID NO: 133 - protein, 13 aa, Artificial Sequence
  CDRH3 dAbH1
TVPGYSTAPYFDL

SEQ ID NO: 134 - protein, 12 aa, Artificial Sequence
  CDRL1 dAbL1
QSSPSVWSNFLS

SEQ ID NO: 135 - protein, 7 aa, Artificial Sequence
  CDRL2 dAbL1
EASKLTS

SEQ ID NO: 136 - protein, 11 aa, Artificial Sequence
  CDRL3 dAbL1
GGGYSSISDTT

SEQ ID NO: 137 - protein, 121 aa, Artificial Sequence
  Heavy chain variable domain of anti-albumin antibody (no ds)
EVQLLESGGGLVQPGGSLRLSCAVSGIDLSNYAINWVRQAPGKGLEWIGIIWASGTTFYATWAKGRFTISRDNSKNTVYLQMNSLRAEDTAVYYCARTVPGYSTAPYFDLWGQGTLVTVSS

SEQ ID NO: 138 - protein, 121 aa, Artificial Sequence
  Heavy chain variable domain of anti-albumin antibody (ds)
EVQLLESGGGLVQPGGSLRLSCAVSGIDLSNYAINWVRQAPGKCLEWIGIIWASGTTFYATWAKGRFTISRDNSKNTVYLQMNSLRAEDTAVYYCARTVPGYSTAPYFDLWGQGTLVTVSS

SEQ ID NO: 139 - protein, 110 aa, Artificial Sequence
  Light chain variable domain of anti-albumin antibody (no ds)
DIQMTQSPSSVSASVGDRVTITCQSSPSVWSNFLSWYQQKPGKAPKLLIYEASKLTSGVPSRFSGSGSGTDFTLTISSLQPEDFATYYCGGGYSSISDTTFGGGTKVEIK

SEQ ID NO: 140 - protein, 112 aa, Artificial Sequence
  Light chain variable domain of anti-albumin antibody (ds)
DIQMTQSPSSVSASVGDRVTITCQSSPSVWSNFLSWYQQKPGKAPKLLIYEASKLTSGVPSRFSGSGSGTDFTLTISSLQPEDFATYYCGGGYSSISDTTFGCGTKVEIKRT

SEQ ID NO: 141 - protein, 1304 aa, Artificial Sequence
  Human CD45
MYLWLKLLAFGFAFLDTEVFVTGQSPTPSPTGLTTAKMPSVPLSSDPLPTHTTAFSPASTFERENDFSETTTSLSPDNTSTQVSPDSLDNASAFNTTGVSSVQTPHLPTHADSQTPSAGTDTQTFSGSAANAKLNPTPGSNAISDVPGERSTASTFPTDPVSPLTTTLSLAHHSSAALPARTSNTTITANTSDAYLNASETTTLSPSGSAVISTTTIATTPSKPTCDEKYANITVDYLYNKETKLFTAKLNVNENVECGNNTCTNNEVHNLTECKNASVSISHNSCTAPDKTLILDVPPGVEKFQLHDCTQVEKADTTICLKWKNIETFTCDTQNITYRFQCGNMIFDNKEIKLENLEPEHEYKCDSEILYNNHKFTNASKIIKTDFGSPGEPQIIFCRSEAAHQGVITWNPPQRSFHNFTLCYIKETEKDCLNLDKNLIKYDLQNLKPYTKYVLSLHAYIIAKVQRNGSAAMCHFTTKSAPPSQVWNMTVSMTSDNSMHVKCRPPRDRNGPHERYHLEVEAGNTLVRNESHKNCDFRVKDLQYSTDYTFKAYFHNGDYPGEPFILHHSTSYNSKALIAFLAFLIIVTSIALLVVLYKIYDLHKKRSCNLDEQQELVERDDEKQLMNVEPIHADILLETYKRKIADEGRLFLAEFQSIPRVFSKFPIKEARKPFNQNKNRYVDILPYDYNRVELSEINGDAGSNYINASYIDGFKEPRKYIAAQGPRDETVDDFWRMIWEQKATVIVMVTRCEEGNRNKCAEYWPSMEEGTRAFGDVVVKINQHKRCPDYIIQKLNIVNKKEKATGREVTHIQFTSWPDHGVPEDPHLLLKLRRRVNAFSNFFSGPIVVHCSAGVGRTGTYIGIDAMLEGLEAENKVDVYGYVVKLRRQRCLMVQVEAQYILIHQALVEYNQFGETEVNLSELHPYLHNMKKRDPPSEPSPLEAEFQRLPSYRSWRTQHIGNQEENKSKNRNSNVIPYDYNRVPLKHELEMSKESEHDSDESSDDDSDSEEPSKYINASFIMSYWKPEVMIAAQGPLKETIGDFWQMIFQRKVKVIVMLTELKHGDQEICAQYWGEGKQTYGDIEVDLKDTDKSSTYTLRVFELRHSKRKDSRTVYQYQYTNWSVEQLPAEPKELISMIQVVKQKLPQKNSSEGNKHHKSTPLLIHCRDGSQQTGIFCALLNLLESAETEEVVDIFQVVKALRKARPGMVSTFEQYQFLYDVIASTYPAQNGQVKKNNHQEDKIEFDNEVDKVKQDANCVNPLGAPEKLPEAKEQAEGSEPTSGTEGPEHSVNGPASPALNQGS

SEQ ID NO: 142 - protein, 226 aa, Artificial Sequence
  Human CD79a
MPGGPGVLQALPATIFLLFLLSAVYLGPGCQALWMHKVPASLMVSLGEDAHFQCPHNSSNNANVTWWRVLHGNYTWPPEFLGPGEDPNGTLIIQNVNKSHGGIYVCRVQEGNESYQQSCGTYLRVRQPPPRPFLDMGEGTKNRIITAEGIILLFCAVVPGTLLLFRKRWQNEKLGLDAGDEYEDENLYEGLNLDDCSMYEDISRGLQGTYQDVGSLNIGDVQLEKP

SEQ ID NO: 143 - protein, 229 aa, Artificial Sequence
  Human CD79b
MARLALSPVPSHWMVALLLLLSAEPVPAARSEDRYRNPKGSACSRIWQSPRFIARKRGFTVKMHCYMNSASGNVSWLWKQEMDENPQQLKLEKGRMEESQNESLATLTIQGIRFEDNGIYFCQQKCNNTSEVYQGCGTELRVMGFSTLAQLKQRNTLKDGIIMIQTLLIILFIIVPIFLLLDKDDSKAGMEEDHTYEGLDIDQTATYEDIVTLRTGEVKWSVGEHPGQE

SEQ ID NO: 144 - protein, 44 aa, Artificial Sequence
  GCN4(7P14P) sequence
ASGGGRMKQLEPKVEELLPKNYHLENEVARLKKLVGERHHHHHH

SEQ ID NO: 145 - DNA, 132 bp, Artificial Sequence
  GCN4(7P14P) sequence
gctagcggaggcggaagaatgaaacaacttgaacccaaggttgaagaattgcttccgaaaaattatcacttggaaaatgaggttgccagattaaagaaattagttggcgaacgccatcaccatcaccatcac

SEQ ID NO: 146 - protein, 262 aa, Artificial Sequence
  52SR4 ds scFv sequence
DAVVTQESALTSSPGETVTLTCRSSTGAVTTSNYASWVQEKPDHLFTGLIGGTNNRAPGVPARFSGSLIGDKAALTITGAQTEDEAIYFCVLWYSDHWVFGCGTKLTVLGGGGGSGGGGSGGGGSGGGGSDVQLQQSGPGLVAPSQSLSITCTVSGFLLTDYGVNWVRQSPGKCLEWLGVIWGDGITDYNSALKSRLSVTKDNSKSQVFLKMNSLQSGDSARYYCVTGLFDYWGQGTTLTVSSAAAHHHHHHEQKLISEEDL

SEQ ID NO: 147 - DNA, 792 bp, Artificial Sequence
  52SR4 ds scFv sequence
gatgcggtggtgacccaggaaagcgcgctgaccagcagcccgggcgaaaccgtgaccctgacctgccgcagcagcaccggcgcggtgaccaccagcaactatgcgagctgggtgcaggaaaaaccggatcatctgtttaccggcctgattggcggcaccaacaaccgcgcgccgggcgtgccggcgcgctttagcggcagcctgattggcgataaagcggcgctgaccattaccggcgcgcagaccgaagatgaagcgatttatttttgcgtgctgtggtatagcgaccattgggtgtttggctgcggcaccaaactgaccgtgctgggtggaggcggtggctcaggcggaggtggctcaggcggtggcgggtctggcggcggcggcagcgatgtgcagctgcagcagagcggcccgggcctggtggcgccgagccagagcctgagcattacctgcaccgtgagcggctttctcctgaccgattatggcgtgaactgggtgcgccagagcccgggcaaatgcctggaatggctgggcgtgatttggggcgatggcattaccgattataacagcgcgctgaaaagccgcctgagcgtgaccaaagataacagcaaaagccaggtgtttctgaaaatgaacagcctgcagagcggcgatagcgcgcgctattattgcgtgaccggcctgtttgattattggggccagggcaccaccctgaccgtgagcagcgcggccgcccatcaccatcaccatcacgaacagaaactgattagcgaagaagatctgtaatag

SEQ ID NO: 148 - protein, 11 aa, Artificial Sequence
  linker sequence
SGGGGSGGGGS

SEQ ID NO: 149 - protein, 8 aa, Artificial Sequence
  Hinge linker Sequence
DKTHTCAA

SEQ ID NO: 150 - protein, 11 aa, Artificial Sequence
  Hinge linker Sequence
DKTHTCPPCPA

SEQ ID NO: 151 - protein, 18 aa, Artificial Sequence
  Hinge linker Sequence
DKTHTCPPCPATCPPCPA

SEQ ID NO: 152 - protein, 25 aa, Artificial Sequence
  Hinge linker Sequence
DKTHTCPPCPATCPPCPATCPPCPA

SEQ ID NO: 153 - protein, 30 aa, Artificial Sequence
  Hinge linker Sequence
DKTHTCPPCPAGKPTLYNSLVMSDTAGTCY

SEQ ID NO: 154 - protein, 31 aa, Artificial Sequence
  Hinge linker Sequence
DKTHTCPPCPAGKPTHVNVSVVMAEVDGTCY

SEQ ID NO: 155 - protein, 15 aa, Artificial Sequence
  Hinge linker Sequence
DKTHTCCVECPPCPA

SEQ ID NO: 156 - protein, 26 aa, Artificial Sequence
  Hinge linker Sequence
DKTHTCPRCPEPKSCDTPPPCPRCPA

SEQ ID NO: 157 - protein, 11 aa, Artificial Sequence
  Hinge linker Sequence
DKTHTCPSCPA

SEQ ID NO: 158 - protein, 7 aa, Artificial Sequence
  Flexible linker sequence
SGGGGSE

SEQ ID NO: 159 - protein, 6 aa, Artificial Sequence
  Flexible linker sequence
DKTHTS

SEQ ID NO: 160 - protein, 6 aa, Artificial Sequence
  Flexible linker sequence
SGGGGS

SEQ ID NO: 161 - protein, 11 aa, Artificial Sequence
  Flexible linker sequence
SGGGGSGGGGS

SEQ ID NO: 162 - protein, 16 aa, Artificial Sequence
  Flexible linker sequence
SGGGGSGGGGSGGGGS

SEQ ID NO: 163 - protein, 21 aa, Artificial Sequence
  Flexible linker sequence
SGGGGSGGGGSGGGGSGGGGS

SEQ ID NO: 164 - protein, 26 aa, Artificial Sequence
  Flexible linker sequence
SGGGGSGGGGSGGGGSGGGGSGGGGS

SEQ ID NO: 165 - protein, 11 aa, Artificial Sequence
  Flexible linker sequence
AAAGSGGASAS

SEQ ID NO: 166 - protein, 16 aa, Artificial Sequence
  Flexible linker sequence
  misc_feature (7)..(7): Xaa can be any naturally occurring amino acid
AAAGSGXGGGSGASAS

SEQ ID NO: 167 - protein, 21 aa, Artificial Sequence
  Flexible linker sequence
  misc_feature (7)..(7): Xaa can be any naturally occurring amino acid
  misc_feature (12)..(12): Xaa can be any naturally occurring amino acid
AAAGSGXGGGSXGGGSGASAS

SEQ ID NO: 168 - protein, 26 aa, Artificial Sequence
  Flexible linker sequence
  misc_feature (7)..(7): Xaa can be any naturally occurring amino acid
  misc_feature (12)..(12): Xaa can be any naturally occurring amino acid
  misc_feature (17)..(17): Xaa can be any naturally occurring amino acid
AAAGSGXGGGSXGGGSXGGGSGASAS

SEQ ID NO: 169 - protein, 31 aa, Artificial Sequence
  Flexible linker sequence
  misc_feature (7)..(7): Xaa can be any naturally occurring amino acid
  misc_feature (12)..(12): Xaa can be any naturally occurring amino acid
  misc_feature (17)..(17): Xaa can be any naturally occurring amino acid
  misc_feature (22)..(22): Xaa can be any naturally occurring amino acid
AAAGSGXGGGSXGGGSXGGGSXGGGSGASAS

SEQ ID NO: 170 - protein, 13 aa, Artificial Sequence
  Flexible linker sequence
  misc_feature (7)..(7): Xaa can be any naturally occurring amino acid
AAAGSGXSGASAS

SEQ ID NO: 171 - protein, 28 aa, Artificial Sequence
  Flexible linker sequence
PGGNRGTTTTRRPATTTGSSPGPTQSHY

SEQ ID NO: 172 - protein, 11 aa, Artificial Sequence
  Flexible linker sequence
ATTTGSSPGPT

SEQ ID NO: 173 - protein, 6 aa, Artificial Sequence
  Flexible linker sequence
ATTTGS

SEQ ID NO: 174 - skipped

SEQ ID NO: 175 - protein, 21 aa, Artificial Sequence
  Flexible linker sequence
EPSGPISTINSPPSKESHKSP

SEQ ID NO: 176 - protein, 15 aa, Artificial Sequence
  Flexible linker sequence
GTVAAPSVFIFPPSD

SEQ ID NO: 177 - protein, 15 aa, Artificial Sequence
  Flexible linker sequence
GGGGIAPSMVGGGGS

SEQ ID NO: 178 - protein, 15 aa, Artificial Sequence
  Flexible linker sequence
GGGGKVEGAGGGGGS

SEQ ID NO: 179 - protein, 15 aa, Artificial Sequence
  Flexible linker sequence
GGGGSMKSHDGGGGS

SEQ ID NO: 180 - protein, 15 aa, Artificial Sequence
  Flexible linker sequence
GGGGNLITIVGGGGS

SEQ ID NO: 181 - protein, 15 aa, Artificial Sequence
  Flexible linker sequence
GGGGVVPSLPGGGGS

SEQ ID NO: 182 - protein, 12 aa, Artificial Sequence
  Flexible linker sequence
GGEKSIPGGGGS

SEQ ID NO: 183 - protein, 18 aa, Artificial Sequence
  Flexible linker sequence
RPLSYRPPFPFGFPSVRP

SEQ ID NO: 184 - protein, 18 aa, Artificial Sequence
  Flexible linker sequence
YPRSIYIRRRHPSPSLTT

SEQ ID NO: 185 - protein, 18 aa, Artificial Sequence
  Flexible linker sequence
TPSHLSHILPSFGLPTFN

SEQ ID NO: 186 - protein, 18 aa, Artificial Sequence
  Flexible linker sequence
RPVSPFTFPRLSNSWLPA

SEQ ID NO: 187 - protein, 18 aa, Artificial Sequence
  Flexible linker sequence
SPAAHFPRSIPRPGPIRT

SEQ ID NO: 188 - protein, 18 aa, Artificial Sequence
  Flexible linker sequence
APGPSAPSHRSLPSRAFG

SEQ ID NO: 189 - protein, 18 aa, Artificial Sequence
  Flexible linker sequence
PRNSIHFLHPLLVAPLGA

SEQ ID NO: 190 - protein, 18 aa, Artificial Sequence
  Flexible linker sequence
MPSLSGVLQVRYLSPPDL

SEQ ID NO: 191 - protein, 18 aa, Artificial Sequence
  Flexible linker sequence
SPQYPSPLTLTLPPHPSL

SEQ ID NO: 192 - protein, 18 aa, Artificial Sequence
  Flexible linker sequence
NPSLNPPSYLHRAPSRIS

SEQ ID NO: 193 - protein, 17 aa, Artificial Sequence
  Flexible linker sequence
LPWRTSLLPSLPLRRRP

SEQ ID NO: 194 - protein, 18 aa, Artificial Sequence
  Flexible linker sequence
PPLFAKGPVGLLSRSFPP

SEQ ID NO: 195 - protein, 18 aa, Artificial Sequence
  Flexible linker sequence
VPPAPVVSLRSAHARPPY

SEQ ID NO: 196 - protein, 17 aa, Artificial Sequence
  Flexible linker sequence
LRPTPPRVRSYTCCPTP

SEQ ID NO: 197 - protein, 18 aa, Artificial Sequence
  Flexible linker sequence
PNVAHVLPLLTVPWDNLR

SEQ ID NO: 198 - protein, 18 aa, Artificial Sequence
  Flexible linker sequence
CNPLLPLCARSPAVRTFP

SEQ ID NO: 199 - protein, 11 aa, Artificial Sequence
  linker sequence
GAPAPAAPAPA

SEQ ID NO: 200 - protein, 4 aa, Artificial Sequence
  linker sequence
PPPP

SEQ ID NO: 201 - protein, 11 aa, Artificial Sequence
  Linker Sequences
DLCLRDWGCLW

SEQ ID NO: 202 - protein, 11 aa, Artificial Sequence
  Linker Sequences
DICLPRWGCLW

SEQ ID NO: 203 - protein, 15 aa, Artificial Sequence
  Linker Sequences
MEDICLPRWGCLWGD

SEQ ID NO: 204 - protein, 20 aa, Artificial Sequence
  Linker Sequences
QRLMEDICLPRWGCLWEDDE

SEQ ID NO: 205 - protein, 20 aa, Artificial Sequence
  Linker Sequences
QGLIGDICLPRWGCLWGRSV

SEQ ID NO: 206 - protein, 21 aa, Artificial Sequence
  Linker Sequences
QGLIGDICLPRWGCLWGRSVK

SEQ ID NO: 207 - protein, 15 aa, Artificial Sequence
  Linker Sequences
EDICLPRWGCLWEDD

SEQ ID NO: 208 - protein, 18 aa, Artificial Sequence
  Linker Sequences
RLMEDICLPRWGCLWEDD

SEQ ID NO: 209 - protein, 16 aa, Artificial Sequence
  Linker Sequences
MEDICLPRWGCLWEDD

SEQ ID NO: 210 - protein, 15 aa, Artificial Sequence
  Linker Sequences
MEDICLPRWGCLWED

SEQ ID NO: 211 - protein, 18 aa, Artificial Sequence
  Linker Sequences
RLMEDICLARWGCLWEDD

SEQ ID NO: 212 - protein, 20 aa, Artificial Sequence
  Linker Sequences
EVRSFCTRWPAEKSCKPLRG

SEQ ID NO: 213 - protein, 20 aa, Artificial Sequence
  Linker Sequences
RAPESFVCYWETICFERSEQ

SEQ ID NO: 214 - protein, 11 aa, Artificial Sequence
  Linker Sequences
EMCYFPGICWM

SEQ ID NO: 215 - protein, 11 aa, Artificial Sequence
  linker sequence
SGGGGTGGGGS